European Patent Specification EP 3 501 535 B1, published September 20, 2023. Title: A METHOD FOR PREVENTION OR TREATMENT OF PORCINE EPIDEMIC DIARRHEA, VACCINE, AND VACCINE KIT. Applicant: NIPPON INSTITUTE FOR BIOLOGICAL SCIENCE. The sequence listing filed with the application follows.

SEQUENCE LISTING (20 sequences)

SEQ ID NO: 1 - DNA, 23 bp, artificial sequence
  1-F primer
gtggcttttctaatcatttggtc

SEQ ID NO: 2 - DNA, 23 bp, artificial sequence
  1-R primer
gcactagtaacattaagcatgta

SEQ ID NO: 3 - DNA, 18 bp, artificial sequence
  2-F primer
ttgtcggcataacatggg

SEQ ID NO: 4 - DNA, 24 bp, artificial sequence
  2-R primer
gttgtaagtatccactttaagaaa

SEQ ID NO: 5 - DNA, 20 bp, artificial sequence
  3-F primer
aaggctcaattgtacttcat

SEQ ID NO: 6 - DNA, 22 bp, artificial sequence
  3-R primer
tcaacacagaaagaactaaacc

SEQ ID NO: 7 - DNA, 21 bp, artificial sequence
  4-F primer
cagccaatttcttttgttact

SEQ ID NO: 8 - DNA, 20 bp, artificial sequence
  4-R primer
tgctctgaaaaagaacatgg

SEQ ID NO: 9 - DNA, 20 bp, artificial sequence
  5-F primer
acatctgattctggacagtt

SEQ ID NO: 10 - DNA, 21 bp, artificial sequence
  5-R primer
agaccttttttgtaccaccct

SEQ ID NO: 11 - DNA, 22 bp, artificial sequence
  6-F primer
atttctgaagaggctctacagt

SEQ ID NO: 12 - DNA, 20 bp, artificial sequence
  6-R primer
ctagaaatggcttggaagtt

SEQ ID NO: 13 - DNA, 20 bp, artificial sequence
  7-F primer
ctcatgcgcttactaaggtt

SEQ ID NO: 14 - DNA, 21 bp, artificial sequence
  7-R primer
catcgatgtaatctgggatta

SEQ ID NO: 15 - DNA, 22 bp, artificial sequence
  8-F primer
cctagaaaacctaccgttagtg

SEQ ID NO: 16 - DNA, 20 bp, artificial sequence
  8-R primer
agctccaactcttggacagc

SEQ ID NO: 17 - DNA, 22 bp, artificial sequence
  9-F primer
gatatgtttgtaatggtaactc

SEQ ID NO: 18 - DNA, 21 bp, artificial sequence
  9-R primer
agcatagctaaaaggcaatgc

SEQ ID NO: 19 - DNA, 22 bp, artificial sequence
  10-F primer
cgcaaagactgaacccactaac

SEQ ID NO: 20 - DNA, 24 bp, artificial sequence
  10-R primer
ttgcctctgttgttacttggagat